European Patent Application EP 4 610 268 A1, published September 3, 2025. Title: Cell-permeable peptides for conjugation. Applicant: AGC Inc. Application JP. The sequence listing filed with the application follows.

SEQUENCE LISTING (1 sequence)

SEQ ID NO: 1 - DNA, 19 bp, synthetic construct
  source 1..19: mol_type = other DNA
tttttcagttgaccatata